European Patent Specification EP 4 069 371 B1, published June 3, 2026. Title: TOOLS AND METHODS TO DETECT AND ISOLATE COLIBACTIN PRODUCING BACTERIA. Applicant: CONSEJO SUPERIOR DE INVESTIGACIONES CIENTIFICAS (CSIC) FUNDACION CIENTIFICA DE LA ASOCIACION ESPAÑOLA CONTRA EL CANCER. Application EP20816209.9. The sequence listing filed with the application follows.

SEQUENCE LISTING (11 sequences)

SEQ ID NO: 1 - protein, 20 aa, Artificial Sequence
  Isolated peptide from colibactinH protein
LDDHGNPVADGEEGELYLAG

SEQ ID NO: 2 - protein, 20 aa, Artificial Sequence
  Isolated peptide from colibactinH protein
WRDGESQQIHYIGRNDFQIK

SEQ ID NO: 3 - protein, 20 aa, Artificial Sequence
  Isolated peptide from colibactinC protein
AAGDRIYAVIRGSAVNNDGK

SEQ ID NO: 4 - protein, 20 aa, Artificial Sequence
  Isolated peptide from colibactinB protein
FNTLVVLENYPVDMTLLSCA

SEQ ID NO: 5 - protein, 1599 aa, Escherichia coli
MEQQGIMRQLPTDDQTIVDYLYRIAGEYGEKAAVLMGDAALSYHDLNARSNQLAHYLRGLGIGEDRVVAIRLPRGMAMLIAIFAIVKAGGAYLPLAYNAPPRSRIENILSNSGAVCLIGTDDGDRWPIPRVEIDSAAVSAMPTTDLRYRPHARQLAYIIYTSGSTGVPKGVATEHAALLNRIVWMQNAYPISSQDVLFQKTVYTFDVSVWEMFWWAMYGASVVLLPSGLESDPRTLARLIQRHRVSVVHFVPSMLNLFVEYLEMKQDPRLTASLRLVFSSGEKLTVHSVARFYQSVAQGDLINLYGPTEAAIDVSHHRCLRGYDYDDIPIGQAIDGCRLYVLDDHGNPVADGEEGELYLAGIGLARGYLNNVALTDRCFTIHPTLRHLGKPERLYKTGDLVWRDGESQQIHYIGRNDFQIKIRGLRVELGEIEAHAMRFPGVQQAVVVADQDDPDNQLIYAFVVSSVPLNLAALMDALSKNLPAYMLPNRLLAMSELPLSDNGKCCRKTLLDLARAYSASRVDLRETPAVRYLPLSSAQSSMWFMQQLAPHTALYNNPTALLLEGELDRTRMDGAIRQLMSRHTLLRAMAETHNGQPVLAVPQCVSSQALLTIVPLPSVSDDNALQAMINQRAAHPMPLTSGTPLCRFELLTLDDDRSVLLIHLHHIISDGWSKGVLLRELQAAYNGESLTPEPLLEYADYMEYQEEWRQSDAYQDAMRYWQNTLAGTLPILDIPTDQPRQKVARYQGAFVAFALSANTCERVLAAARAQRVSLYNYLLTAFVLLLHRNARQQEYIVGMPIAARLTKEQEHMIAPLVNVLPLRLPLDEAASFSELVQTIRGILFAAFRHQRLEFTDIVRAVNVDRSAGHFPIYQCMFQLDNMPLASPTLNGVNVTPLLLDTSASQVDISLSMQHIDGRITGTFEYDAGLYSADRIQHLVAQWRELLDEASSQPTQLVRDLIRFTPREHAWLARHNATEVALPPVDNLLALVLPHCQQRPTQVALRHADDAMTYGELQQATMQMCTWLRAQGVKRGESVALQLPFCFELIIAQLAILSLGASYVPLDGNAPAARNALILAQATPCMLLVAQPLESPHGLTIPWVLVPDWRSLLTEIPNLPVSVAPDALDCDAVVIFTSGTTGQPKGVRLSQRNLVNLTASFISSYQVTHQDVLLPITSVASASFVGEVLPLLAAGGTLVLAQKAQSLDSDALIALLASQRVTILSTTPSLSASLSVLAQSMGSLRLFLCGGEALEYEQIAPLLPHMAVVNGYGLTESGICSTYFPVAKRREQETGALPIGRPIQNTQAYVVDAYNRLVPPGACGELCFSGLGISPGYLDARQDPERFVELPEYPGVRVLKTGDRARWATDGMLFYLGRQDRQVQIRGYRVELGDIESLLKQHPDIADAWVDVRRNAAATPLLVAFYCSVNGVALDAQQLRVWLSLRLPLHMLPLLYVPLSAMPLGVNGKIDPQCLPLVDLRQLEGPGEYVPPATELEQRLAEIWQQLLGLERVGTTTNFFDLGGHSLLLVQMQQYIGQQCGQHVALVDLLRFTTIKRLAEFLLAPDAAQGTTGDQTQLRAAKQRLAFGHTRWAATTDSHH

SEQ ID NO: 6 - protein, 866 aa, Escherichia coli
MEYASEMNGMEIAIIGMAVRFPQSRTLHEFWHNIVQGKECVTFFSEEELLAEGVEQSTLDNPAYVRAKPYIKGICDFDAAFFGYSHKEAQTLDPKSRVLHEVAYHALEDAGYAQRTSDLITGVFVGASEDVDWLRRSLSQIGGDALNRFESGIYGHKDLLAHLIAYSLNLNGPVYSLYTSCSTSLSATHIACRSLLFGECDLALAGGITIDLPQKSGYFCQQGMIHSTDGHCRPFDSQASGTLFGDGAGVVVLRRLEDALAAGDRIYAVIRGSAVNNDGKQKIGFVAPGHEGQKAVICAACHLAEVSPESIGYVETHGTGTRIGDLIEFAALTEAFDTSHRQYCALGAVKANIGHTHAAAGVAGLIKTALVLHHRTIPPLANYQMPNSKLDLAHSPFYIPIQPQEWPASRMPPRAGVSSFGIGGTNVHMILEGLNPAVRDDHDQVRAPVFIPLSAPSFEQLDELTQQLTPLLATLDASTLAYTQQVARPVFDCRRVIQVENDGTQAMLASLDNLMPDAPWGLHCPDLRTTNDCTYAQWLAHSAHYQREATALTALLDGMNIPPAYCHAETWAAQANSSLLIRGCQTIAALKTWMNLLPTLTLLSGAGTGLLPAAAASGMIATQDVLHLLWEMEQKALHLWLPERHEPIPGYVLAWQGNPITDAQRNDRGFWSEALLADTRELGEGVHSINWVRLPPEIREDVDVLRYVAQLWCAGINVDWAVWYGTPLPQRGSASAYPFAHNHYPLPGRVMGSVETQPEAGPETHHPYQARPVLSVPFVAAHSRGMQYITGLMELLLEISPVGVDDDFFELGGHSLLVTQLTSRLERDFNVHIDLLTLMENPNPRNIYAHIAAQLGGEDNLEIACQ

SEQ ID NO: 7 - skipped

SEQ ID NO: 8 - DNA, 21 bp, Artificial Sequence
  ClbB1 reverse primer 1
ccatttcccgtttgagcacac

SEQ ID NO: 9 - DNA, 23 bp, Artificial Sequence
  clbB1 forward primer 1
gatttggatactggcgataaccg

SEQ ID NO: 10 - DNA, 20 bp, Artificial Sequence
  clbB2 reverse primer 1
gcgctctatgctcatcaacc

SEQ ID NO: 11 - DNA, 21 bp, Artificial Sequence
  clbB2 forward primer 1
gcgcatcctcaagagtaaata